European Patent Application EP 4 631 524 A2, published October 15, 2025. Title: COMBINATION COMPRISING AN ADC OR AN AOC COMPRISING A VHH, AND A SAPONIN OR A LIGAND-SAPONIN CONJUGATE. Applicant: Sapreme B.V. Application EP. The sequence listing filed with the application follows.

SEQUENCE LISTING (72 sequences)

SEQ ID NO: 1 - DNA, 414 bp, Camelus dromedarius
  source 1..414: mol_type = other DNA
gaagttcagctgcaggaatctggtggtggtctggttcagccgggtggttctctgcgtctgtcttgcgcggcgtctggtttcatcttctctaacgacgcgatgacctgggttcgtcaggcgccgggtaaaggtctggaatgggtttcttctatcaactggtctggtacccacaccaactacgcggactctgttaaaggtcgtttcaccatctctcgtgacaacgcgaaacgtaccctgtacctgcagatgaactctctgaaagacgaagacaccgcgctgtactactgcgttaccggttacggtgttaccaaaaccccgaccggtcagggtacccaggttaccgtttcttctcaccaccaccaccaccactctccgtctaccccgccgaccccgtctccgtctaccccgccgtgc

SEQ ID NO: 2 - protein, 138 aa, Camelus dromedarius
EVQLQESGGGLVQPGGSLRLSCAASGFIFSNDAMTWVRQAPGKGLEWVSSINWSGTHTNYADSVKGRFTISRDNAKRTLYLQMNSLKDEDTALYYCVTGYGVTKTPTGQGTQVTVSSHHHHHHSPSTPPTPSPSTPPC

SEQ ID NO: 3 - DNA, 375 bp, Camelus dromedarius
  source 1..375: mol_type = other DNA
atggaagttcagctggttgaatctggtggtggtctggttcaggcgggtggttctctgcgtctgtcttgcgcggcgtctggtatcaccttctctatcaacaccatgggttggtaccgtcaggcgccgggtaaacagcgtgaactggttgcgctgatctcttctatcggtgacacctactacgcggactctgttaaaggtcgtttcaccatctctcgtgacaacgcgaaaaacaccgtttacctgcagatgaactctctgaaaccggaagacaccgcggtttactactgcaaacgtttccgtaccgcggcgcagggtaccgactactggggtcagggtacccaggttaccgtttcttctcaccaccaccaccaccac

SEQ ID NO: 4 - protein, 125 aa, Camelus dromedarius
MEVQLVESGGGLVQAGGSLRLSCAASGITFSINTMGWYRQAPGKQRELVALISSIGDTYYADSVKGRFTISRDNAKNTVYLQMNSLKPEDTAVYYCKRFRTAAQGTDYWGQGTQVTVSSHHHHHH

SEQ ID NO: 5 - DNA, 375 bp, synthetic construct
  source 1..375: mol_type = other DNA; note = Amino-acid coding DNA sequence of Anti-HER2 dsAb pcNB2
atggaagttcagctggttgaaaaaggtggtggtcgtgttcaggcgggtggttctctgcgtctgcgttgcgcggcgtctggtatcaccttctctatcaacaccatgggttggtaccgtcaggcgccgggtaaacagcgtgaactggttgcgctgatctcttctatcggtgacacctactacgcggactctgttaaaggtcgtttccgtatccgtcgtgacaacgcgaaaaacaccgtttacctgcgtatgcgtcgtctgaaaccggaagacaccgcggtttactactgcaaacgtttccgtaccgcggcgcagggtaccgactactggggtcagggtacccgtgttaccgtttctaaacaccaccaccaccaccac

SEQ ID NO: 6 - protein, 125 aa, synthetic construct
  source 1..125: note = Amino-acid sequence of Anti-HER2 dsAb pcNB2
MEVQLVEKGGGRVQAGGSLRLRCAASGITFSINTMGWYRQAPGKQRELVALISSIGDTYYADSVKGRFRIRRDNAKNTVYLRMRRLKPEDTAVYYCKRFRTAAQGTDYWGQGTRVTVSKHHHHHH

SEQ ID NO: 7 - DNA, 378 bp, Camelus dromedarius
  source 1..378: mol_type = other DNA
gcggcgcaggttaaactggaagaatctggtggtggttctgttcagaccggtggttctctgcgtctgacctgcgcggcgtctggtcgtacctctcgttcttacggtatgggttggttccgtcaggcgccgggtaaagaacgtgaattcgtttctggtatctcttggcgtggtgactctaccggttacgcggactctgttaaaggtcgtttcaccatctctcgtgacaacgcgaaaaacaccgttgacctgcagatgaactctctgaaaccggaagacaccgcgatctactactgcgcggcggcggcgggttctgcgtggtacggtaccctgtacgaatacgactactggggtcagggtacccaggttaccgtttcttct

SEQ ID NO: 8 - protein, 126 aa, Camelus dromedarius
AAQVKLEESGGGSVQTGGSLRLTCAASGRTSRSYGMGWFRQAPGKEREFVSGISWRGDSTGYADSVKGRFTISRDNAKNTVDLQMNSLKPEDTAIYYCAAAAGSAWYGTLYEYDYWGQGTQVTVSS

SEQ ID NO: 9 - DNA, 381 bp, Camelus dromedarius
  source 1..381: mol_type = other DNA
gaagttcagctggttgaatctggtggtggtctggttcaggcgggtggttctctgcgtctgtcttgcgcggcgtctggtcgtaccttctcttcttacgcgatgggttggttccgtcaggcgccgggtaaagaacgtgaattcgttgttgcgatcaactggtcttctggttctacctactacgcggactctgttaaaggtcgtttcaccatctctcgtgacaacgcgaaaaacaccatgtacctgcagatgaactctctgaaaccggaagacaccgcggtttactactgcgcggcgggttaccagatcaactctggtaactacaacttcaaagactacgaatacgactactggggtcagggtacccaggttaccgtttcttct

SEQ ID NO: 10 - protein, 127 aa, Camelus dromedarius
EVQLVESGGGLVQAGGSLRLSCAASGRTFSSYAMGWFRQAPGKEREFVVAINWSSGSTYYADSVKGRFTISRDNAKNTMYLQMNSLKPEDTAVYYCAAGYQINSGNYNFKDYEYDYWGQGTQVTVSS

SEQ ID NO: 11 - DNA, 378 bp, synthetic construct
  source 1..378: mol_type = other DNA; note = Amino-acid coding DNA sequence of Anti-VGFR2 dsAb NTV1
atggcgcaggttcagctgctggaatctggtggtggtctggttcagccgggtggttctctgcgtctgtcttgcgcggcgtctggttactctgttatcaacgacttcatgacctgggttcgtcaggcgccgggtaaaggtctggaatgggtttcttctatctctgttgcggacggttctacctactacgcggactctgttaaaggtcgtttcaccatctctcgtgacaactctaaaaacaccctgtacctgcagatgaactctctgcgtgcggaagacaccgcggtttactactgcgcggcgcgtgttggtggtcgtgacctgggttggccgtacgaactggactactggggtcagggtaccctggttaccgtttcttct

SEQ ID NO: 12 - protein, 126 aa, synthetic construct
  source 1..126: note = Amino-acid sequence of Anti-VGFR2 dsAb NTV1
MAQVQLLESGGGLVQPGGSLRLSCAASGYSVINDFMTWVRQAPGKGLEWVSSISVADGSTYYADSVKGRFTISRDNSKNTLYLQMNSLRAEDTAVYYCAARVGGRDLGWPYELDYWGQGTLVTVSS

SEQ ID NO: 13 - DNA, 372 bp, synthetic construct
  source 1..372: mol_type = other DNA; note = Amino-acid coding DNA sequence of Anti-VGFR2 dsAb NTV2
atggcgcaggttcagctgctggaatctggtggtggtctggttcagccgggtggttctctgcgtctgtcttgcgcggcgtctggtttcaaaatcaccaacaaaaccatggcgtgggttcgtcaggcgccgggtaaaggtctggaatgggtttcttctatcggttcttcttctggttctacctactacgcggactctgttaaaggtcgtttcaccatctctcgtgacaactctaaaaacaccctgtacctgcagatgaactctctgcgtgcggaagacaccgcggtttactactgcgcgcgtcgtaaaggtaaccgtctgggtccggcggcgctgcgttcttggggtcagggtaccctggttaccgtttcttct

SEQ ID NO: 14 - protein, 124 aa, synthetic construct
  source 1..124: note = Amino-acid sequence of Anti-VGFR2 dsAb NTV2
MAQVQLLESGGGLVQPGGSLRLSCAASGFKITNKTMAWVRQAPGKGLEWVSSIGSSSGSTYYADSVKGRFTISRDNSKNTLYLQMNSLRAEDTAVYYCARRKGNRLGPAALRSWGQGTLVTVSS

SEQ ID NO: 15 - DNA, 363 bp, synthetic construct
  source 1..363: mol_type = other DNA; note = Amino-acid coding DNA sequence of Anti-VGFR2 dsAb NTV3
atggcgcaggttcagctgctggaatctggtggtggtctggttcagccgggtggttctctgcgtctgtcttgcgcggcgtctggtgttcgtgttaactacaaatctatgtcttgggttcgtcaggcgccgggtaaaggtctggaatgggtttctaccatcacctctcgtaacggttctacctactacgcggactctgttaaaggtcgtttcaccatctctcgtgacaactctaaaaacaccctgtacctgcagatgaactctctgcgtgcggaagacaccgcggtttactactgcgcgaccggtcgtgcgcaccacgcgccggttcgttactggggtcagggtaccctggttaccgtttcttct

SEQ ID NO: 16 - protein, 121 aa, synthetic construct
  source 1..121: note = Amino-acid sequence of Anti-VGFR2 dsAb NTV3
MAQVQLLESGGGLVQPGGSLRLSCAASGVRVNYKSMSWVRQAPGKGLEWVSTITSRNGSTYYADSVKGRFTISRDNSKNTLYLQMNSLRAEDTAVYYCATGRAHHAPVRYWGQGTLVTVSS

SEQ ID NO: 17 - DNA, 363 bp, synthetic construct
  source 1..363: mol_type = other DNA; note = Amino-acid coding DNA sequence of Anti-VGFR2 dsAb NTV4
atggcgcaggttcagctgctggaatctggtggtggtctggttcagccgggtggttctctgcgtctgtcttgcgcggcgtctggtgttaccatcaccgacgaagacatgacccgtgttcgtcaggcgccgggtaaaggtctggaatgggtttcttctatcctgaacaccggtggttctacctactacgcggactctgttaaaggtcgtttcaccatctctcgtgacaactctaaaaacaccctgtacctgcagatgaactctctgcgtgcggaagacaccgcggtttactactgcgcggcggttcacgaaaaagcggcggacatgaacttctggggtcagggtaccctggttaccgtttcttct

SEQ ID NO: 18 - protein, 120 aa, synthetic construct
  source 1..120: note = Amino-acid sequence of Anti-VGFR2 dsAb NTV4
AQVQLLESGGGLVQPGGSLRLSCAASGVTITDEDMTRVRQAPGKGLEWVSSILNTGGSTYYADSVKGRFTISRDNSKNTLYLQMNSLRAEDTAVYYCAAVHEKAADMNFWGQGTLVTVSS

SEQ ID NO: 19 - DNA, 327 bp, Camelus bactrianus
  source 1..327: mol_type = other DNA
gaagttcagctgctggaatctggtggtggtctggttcagccgggtggttctctgcgttcttgcgaagcgtctggtttcaacgcgatgacctctatcgactcttggaccgacgcggttaaaggttgggttcgtcagccgccgggtaaaggtctggaatgggtttctcgtttcgcgatctctcaggacaacgcgaaaaacaccgtttacctgcagatgaactctctgaaaccggaagacaccgcgatgtactactgcgcgctgtctaaatgctacacccgtgtttacgactactggggtcagggtacccaggttaccgtttcttctggt

SEQ ID NO: 20 - protein, 109 aa, Camelus bactrianus
EVQLLESGGGLVQPGGSLRSCEASGFNAMTSIDSWTDAVKGWVRQPPGKGLEWVSRFAISQDNAKNTVYLQMNSLKPEDTAMYYCALSKCYTRVYDYWGQGTQVTVSSG

SEQ ID NO: 21 - DNA, 312 bp, Camelus bactrianus
  source 1..312: mol_type = other DNA
gaagttcagctgcaggaatctggtggtggtctggttcagccgggtggttctctgcgtctgtcttgcgcggcgtctggtttcatctacatggttggtatcaaaaccgaacgtgacggtgttaaaggttgggttcgtcaggcgccgggtaaaggtctggaatggctgtctcgtttcaccatcccgcgtgacaacgcgaaaaacaccctgtacctgcagatgaacaacctgaaatctgaagacaccgcgctgtactactgcgcgaccgaagaaaacgactggggtcagggtacccaggttaccgtttcttctggt

SEQ ID NO: 22 - protein, 104 aa, Camelus bactrianus
EVQLQESGGGLVQPGGSLRLSCAASGFIYMVGIKTERDGVKGWVRQAPGKGLEWLSRFTIPRDNAKNTLYLQMNNLKSEDTALYYCATEENDWGQGTQVTVSSG

SEQ ID NO: 23 - DNA, 351 bp, Camelus dromedarius
  source 1..351: mol_type = other DNA
caggttcagctgcaggaatctggtggtggttctgttcaggcgggtggttctctgcgtctgtcttgcaccgcgtctggtttcggtgttgacggtaccgacatgggttggtaccgtcaggcgccgggtaacgaatgcgaactggtttcttctatctcttctatcggtatcggttactactctgaatctgttaaaggtcgtttcaccatctctcgtgacaacgcgaaaaacaccgtttacctgcagatgaactctctgcgtccggacgacaccgcggtttactactgcggtcgtcgttggatcggttaccgttgcggtaactggggtcgtggtacccaggttaccgtttcttct

SEQ ID NO: 24 - protein, 117 aa, Camelus dromedarius
QVQLQESGGGSVQAGGSLRLSCTASGFGVDGTDMGWYRQAPGNECELVSSISSIGIGYYSESVKGRFTISRDNAKNTVYLQMNSLRPDDTAVYYCGRRWIGYRCGNWGRGTQVTVSS

SEQ ID NO: 25 - DNA, 369 bp, Camelus dromedarius
  source 1..369: mol_type = other DNA
caggttcagctgcaggaatctggtggtggttctgttcaggcgggtggttctctgcgtctgtcttgcaccggttctcgttacacctacaccatgggttggttccgtcaggcgccgggtaaagaacgtgaaggtgttgttgcgatcaccgcgttcggttctccgttctacgcggactctgttaaaggtcgtttcaccatctctcgtgacaacgcgaacaacaccatcttcctgcagatgaactctctgaaaccggaagactctgcgatgtactactgcgcggcgcgtggttcttctggtacctcttacaaatggaacgaatacggttcttacaactactggggtcagggtacccaggttaccgtttcttct

SEQ ID NO: 26 - protein, 123 aa, Camelus dromedarius
QVQLQESGGGSVQAGGSLRLSCTGSRYTYTMGWFRQAPGKEREGVVAITAFGSPFYADSVKGRFTISRDNANNTIFLQMNSLKPEDSAMYYCAARGSSGTSYKWNEYGSYNYWGQGTQVTVSS

SEQ ID NO: 27 - DNA, 351 bp, Camelus dromedarius
  source 1..351: mol_type = other DNA
caggttcagctgcaggaatctggtggtggttctgttcaggcgggtggttctctgcgtctgtcttgcgcggcgtctaaatacacctcttgcatgggttggttccgtcaggcgccgggtaaagaacgtgaagttgttgcgcacatcgactctggtccgcgtaccctgtacgcggactctgttaaaggtcgtttcaccatctctaaagacaacgcgaaaaacaccctgtacctggaaatgtctaccctgaaaccggacgacaccgcgatgtactactgcgcggcgggtccgatgtactctggttcttgcaactacaactactggggtcagggtacccaggttaccgtttcttct

SEQ ID NO: 28 - protein, 117 aa, Camelus dromedarius
QVQLQESGGGSVQAGGSLRLSCAASKYTSCMGWFRQAPGKEREVVAHIDSGPRTLYADSVKGRFTISKDNAKNTLYLEMSTLKPDDTAMYYCAAGPMYSGSCNYNYWGQGTQVTVSS

SEQ ID NO: 29 - DNA, 366 bp, Camelus dromedarius
  source 1..366: mol_type = other DNA
caggttcagctgcaggaatctggtggtggtctggttcagccgggtggttctctgcgtctgtcttgcgcggcgtctggtttcaccctggactactacgcgatcggttggttccgtcaggcgccgggtaaagaacgtgaaggtgtttcttgcatctcttcttctgacggttctacctactacgcggactctgttaaaggtcgtttcaccatctctcgtgacaacgcgaaaaacaccgtttacctgcagatgtcttctctgaaaccggaagacaccgcggtttactactgcggtatctctggttcttgcctgctggaagactacggtatggactactggggtaaaggtacccaggttaccgtttcttct

SEQ ID NO: 30 - protein, 122 aa, Camelus dromedarius
QVQLQESGGGLVQPGGSLRLSCAASGFTLDYYAIGWFRQAPGKEREGVSCISSSDGSTYYADSVKGRFTISRDNAKNTVYLQMSSLKPEDTAVYYCGISGSCLLEDYGMDYWGKGTQVTVSS

SEQ ID NO: 31 - DNA, 378 bp, Camelus dromedarius
  source 1..378: mol_type = other DNA
caggttcagctgcaggaatctggtggtggtctggttcacccgggtggttctctgcgtctgtcttgcgcggcgtctggtttctctctggacaactacgcgatcggttggttccgtcaggcgccgggtaaagaacgtgaaggtgtttcttgcatctcttctggttctgaaggtcgtcgttactacgcggacttcgttaaaggtcgtttcaccatctctcgtgacaacgcgaaaaacaccgcgttcctgcagatgaactctctgaaaccggaagacaccgcggactactactgcgcgaccgttggtttctgctcttctcagtacggtatggaattcgttggtgactactggggtcagggtacccaggttaccgtttcttct

SEQ ID NO: 32 - protein, 126 aa, Camelus dromedarius
QVQLQESGGGLVHPGGSLRLSCAASGFSLDNYAIGWFRQAPGKEREGVSCISSGSEGRRYYADFVKGRFTISRDNAKNTAFLQMNSLKPEDTADYYCATVGFCSSQYGMEFVGDYWGQGTQVTVSS

SEQ ID NO: 33 - protein, 115 aa, synthetic construct
  source 1..115: note = Amino-acid sequence of Anti-mouse serum albumin dsAb MSA21
QVQLQESGGGLVQPGGSLRLSCEASGFTFSRFGMTWVRQAPGKGVEWVSGISSLGDSTLYADSVKGRFTISRDNAKNTLYLQMNSLKPEDTAVYYCTIGGSLNPGGQGTQVTVSS

SEQ ID NO: 34 - protein, 115 aa, synthetic construct [sequence omitted]

SEQ ID NO: 35 - protein, 114 aa, synthetic construct
  source 1..114: note = Amino-acid sequence of Anti-human serum albumin dsAb Alb23
EVQLLESGGGLVQPGGSLRLSCAASGFTFRSFGMSWVRQAPGKGPEWVSSISGSGSDTLYADSVKGRFTISRDNSKTLYLQMNSLRPEDTAVYYCTIGGSLSRSSQGTLVTVSS

SEQ ID NO: 36 - protein, 125 aa, synthetic construct
  source 1..125: note = Amino-acid sequence of Anti-EGFR VHH 7A5
EVQLVESGGGLVQAGGSLRLSCAASDRTFSSNNMGWFRQAPGKEREFVAAIGWGGLETHYSDSVKGRFTISRDNAKNTVYLQMNSLKPEDTARYYCAVSSTRTVIYTLPRMYNYWGQGTQVTVSS

SEQ ID NO: 37 - protein, 124 aa, synthetic construct
  source 1..124: note = Amino-acid sequence of Anti-EGFR VHH 7D12
QVKLEESGGGSVQTGGSLRLTCAASGRTSRSYGMGWFRQAPGKEREFVSGISWRGDSTGYADSVKGRFTISRDNAKNTVDLQMNSLKPEDTAIYYCAAAAGSAWYGTLYEYDYWGQGTQVTVSS

SEQ ID NO: 38 - protein, 124 aa, synthetic construct
  source 1..124: note = Amino-acid sequence of Anti-EGFR VHH 7C12
AVQLVESGGGSVQAGGSLRLTCAASGRTSRSYGMGWFRQAPGKEREFVSGISWRGDSTGYADSVKGRFTISRDNAKNTVDLQMNSLKPEDTAIYYCAAAAGSTWYGTLYEYDYWGQGTQVTVSS

SEQ ID NO: 39 - protein, 114 aa, synthetic construct
  source 1..114: note = Amino-acid sequence of Anti-insulin-like growth factor 1 receptor VHH 4B11
EVQLVESGGGLVQPGGSLRLSCAASGSIFTFNAMGWYRQAPGKQRELVAVIISGGSTHYVDSVKGRFTISRDNAKKMVYLQMNSLKPEDTAVYYCNVKKFGDYWGQGTQVTVSS

SEQ ID NO: 40 - protein, 116 aa, synthetic construct
  source 1..116: note = Amino-acid sequence of Anti-insulin-like growth factor 1 receptor VHH 3G7
DVQLVESGGGLVQAGGSLRLSCAASESISTINVMAWYRQAPGKQRELVAEITRSGRTNYVDSVKGRFTISRDNAKNTMYLQMNSLNLEDTAVYYCRTIDGSWREYWGQGTQVTVSS

SEQ ID NO: 41 - protein, 127 aa, synthetic construct
  source 1..127: note = Amino-acid sequence of Anti-insulin-like growth factor 1 receptor VHH 2C7
QVKLEESGGGLVQPGGSLRLSCVASGRTFSNYAIVIGWFRQAPGQEREFVAAINWNSRSTYYADSVKGRFTISRLNARNTVYLQMNRLKPEDTAVYDCAASHDSDYGGTNANLYDYWGQGTQVTVSS

SEQ ID NO: 42 - protein, 124 aa, synthetic construct
  source 1..124: note = Amino-acid sequence of Anti-insulin-like growth factor 1 receptor VHH 1C7
QVKLEESGGGLVQAGGSLRLSCVASGRTFSRTANAWFRQAPGKEREFVATITWNSGTTRYADSVKGRFFISKDSAKNTIYLEMNSLEPEDTAVYYCAATAAAVITPTRGYYNYWGQGTQVTVSS

SEQ ID NO: 43 - protein, 123 aa, synthetic construct
  source 1..123: note = Amino-acid sequence of Anti-CEACAM VHH NbCEA5
EVQLVESGGGSVQAGGSLRLSCAASGDTYGSYWMGWFRQAPGKEREGVAAINRGGGYTVYADSVKGRFTISRDTAKNTVYLQMNSLRPDDTADYYCAASGVLGGLHEDWFNYWGQGTLVTVSS

SEQ ID NO: 44 - protein, 123 aa, synthetic construct
  source 1..123: note = Amino-acid sequence of Anti-CEACAM VHH CEA5
EVQLVESGGGSVQAGGSLRLSCAASGDTYGSYWMGWFRQAPGQEREAVAAINRGGGYTVYADSVKGRFTISRDNAKNTLYLQMNSLRPDDTADYYCAASGVLGGLHEDWFNYWGQGTLVTVSS

SEQ ID NO: 45 - protein, 116 aa, synthetic construct
  source 1..116: note = Amino-acid sequence of Anti-CD123 VHH 57A07
EVQLVESGGGLVQAGGSLRLSCAASGSIFSGNVMGWYRRQAPGKEREWVAAIASGGSIYYRDSVKGRFTISRDNAKNTVYLQMNSLKPEDTAVYYCNSHPPTLPYWGLGTQVTVSS

SEQ ID NO: 46 - protein, 116 aa, synthetic construct
  source 1..116: note = Amino-acid sequence of Anti-CD123 VHH 57B04
EVQLVESGGGLVQPGGSLRLSCAASGINFRFNSMGWWRRRAPGKEREWVAAITSGDITNYRDSVRGRFTISRDNVKNTVYLQMNTLKLEDTAVYYCNTFPPIADYWGLGTQVTVSS

SEQ ID NO: 47 - protein, 123 aa, synthetic construct
  source 1..123: note = Amino-acid sequence of Anti-CD123 VHH 51D09
EVQLVESGGGLVQPGGSLRLSCAASGSIFSGNTMGWYRQAPGKQRELVAAISSGGSTDYADSVKGRFTISRDNSKNTVYLQMNSLRPEDTAVYYCNAAILLYRLYGYEEGDYWGLGTLVTVSS

SEQ ID NO: 48 - protein, 125 aa, synthetic construct
  source 1..125: note = Amino-acid sequence of Anti-CD123 VHH 55C05
EVQLVESGGGLVPAGDSLRLSCVASGRSLNTYTMGWFRQAPGKECEEVAAINWNGVYRDYADSAKGRETASRDNAMNTVFLQMNSLKPEDTAVYFCATATQGWDRHTEPSDFGSWGLGTQVTVSS

SEQ ID NO: 49 - protein, 124 aa, synthetic construct
  source 1..124: note = Amino-acid sequence of Anti-CD123 VHH 50F07
EVQLVESGGGLVQPGGSLRLSCTGSGSTFSINAMGWYRQAPGKQRELVAAITSGGRTNYADSVKGRFTISRDNSKNTVYLQMNSLRPEDTAVYYCNARISAGTAFWLWSDYEYWGLGTLVTVSS

SEQ ID NO: 50 - protein, 125 aa, synthetic construct
  source 1..125: note = Amino-acid sequence of Anti-CD123 VHH 55F03
EVQLVESGGGLVQAGGPLRLSCAASGRTFSSYVMGWFRQAPGKEREFVAAIYWSNGKTQYTDSVKGRFTISGDNAKNTVYLQMNSLNPEDTAVYYCVADKDETGFRTLPIAYDYWGLGTQVTVSS

SEQ ID NO: 51 - protein, 126 aa, synthetic construct
  source 1..126: note = Amino-acid sequence of Anti-CD123 VHH 55A01
EVQLVESGGGSVQAGGSLRLSCTTSGRALNMYVMGWFRQAPGNEREFVAATSSSGGSTSYPDSVKGRFTISRDNAKNTVYLQMNSLKPEDTAAYRCAASPYVSTPTMNILEEYRYWGLGTQVTVSS

SEQ ID NO: 52 - protein, 125 aa, synthetic construct
  source 1..125: note = Amino-acid sequence of Anti-c-MET VHH 04E09
EVQLVESGGGLVQPGGSLRLSCAASGFILDYYAIGWFRQAPGKEREGVLCIDASDDITYYADSVKGRFTISRDNAKNTVYLQMNSLKPEDTGVYYCATPIGLSSSCLLEYDYDYWGQGTLVTVSS

SEQ ID NO: 53 - protein, 130 aa, synthetic construct
  source 1..130: note = Amino-acid sequence of Anti-c-MET VHH 06B08
EVQLVESGGGLVQAGGSLRLSCAASGRTISRYTMGWFRQAPGKEREFVAAISWSGDNTNYADSVKGRFTISRPNTKNTMYLQMNSLKPEDTAVYYCAADYRSGSYYQASEWTRPSGYDYWGQGTLVTVSS

SEQ ID NO: 54 - protein, 125 aa, synthetic construct
  source 1..125: note = Amino-acid sequence of Anti-c-MET VHH 06C12
EVQLVESGGGLVQPGGSLRLSCAASGFSLDYFAIGWFRQAPGKEREEISCISNSDGSTYYANSVKGRFTISIDNAKNTVYLQMTSLKPEDTAVYYCATPVGLGPFCKTTNDYDYSGQGTLVTVSS

SEQ ID NO: 55 - protein, 124 aa, synthetic construct
  source 1..124: note = Amino-acid sequence of Anti-c-MET VHH 06F10
EVQLVESGGGLVQPGGSLRLSCAASGFTLDYYAINWFRQAPGKEREGVSCISGGDGSTYYADSVKGRFTISRDNAKNTVYLQMNSLKPEDTAVYYCATALGLSSSCHGDGYDYWGQGTLVTVSS

SEQ ID NO: 56 - protein, 125 aa, synthetic construct
  source 1..125: note = Amino-acid sequence of Anti-Her3 VHH 21F6
EVQLVESGGGLVQAGGSLRLSCAASGRTYYLNAMGWFRQGPGKDREFVAAIDWSDGNKDYADSVKGRFTISRDNAKNTVYLQMNSLKPEDTAVYYCAADTPPWGPMIYIESYDSWGQGTLVTVSS

SEQ ID NO: 57 - protein, 113 aa, synthetic construct
  source 1..113: note = Amino-acid sequence of Anti-Her3 VHH 4C7
EVQLVESGGGLVQAGGSLRLSCAASGFTFSSYPMSWVRQAPGKGPAWVSTVSPGGITTSYADSVKGRFTISRDNAKNTLYLQMNSLKPEDTAVYYCLRDLNNRGQGTLVTVSS

SEQ ID NO: 58 - protein, 118 aa, synthetic construct
  source 1..118: note = Amino-acid sequence of Anti-Her3 VHH 17B5
EVQLVESGGGLVQPGGSLRLSCAASGSIGGLNAMAWYRQAPGKERELVAGIFGVGSTRYADSVKGRFTISRDIAKNTVFLQMNSLNSEDTAVYYCRMSSVTRGSSDYWGQGTQVTVSS

SEQ ID NO: 59 - protein, 122 aa, synthetic construct
  source 1..122: note = Amino-acid sequence of Anti-Her3 VHH 18G11
EVQLVESGGGLVQPGGSLRLSCAASGTLFKINAMGWYRQAPGKRRELVALITSSDTTDYAESVEGRFTISRDNTWNAVYLQMNSLKPEDTAVYYCHSDHYSMGVPEKRVIMYGQGTQVTVSS

SEQ ID NO: 60 - protein, 120 aa, synthetic construct
  source 1..120: note = Amino-acid sequence of Anti-Her3 VHH 34C7
EVQLVESGGGLVQPGGSLGLSCVASGSIFRINAMAWYRQAPGKQRELVAEITAGGSTNYADSVKGRFTISVDNAWNTLYLQMNSLKVEDTAVYYCNLDHYTTWDRRSAYWGQGTQVTVSS

SEQ ID NO: 61 - protein, 119 aa, Lama glama
KVQLVESGGGLVQPGGSLRLSCAASGSIFGFNDMAWYRQAPGKQRELVALISRVGVTSSADSVKGRFTISRVNAKDTVYLQMNSLKPEDTAVYYCYMDQRLDGSTLAYWGQGTQVTVSS

SEQ ID NO: 62 - protein, 124 aa, Lama glama
EVQLVESGGSLVQPGGSLRLSCAASGFTFDDYAMSWVRQVPGKGLEWVSSINWSGTHTDYADSVKGRFTISRNNANNTLYLQMNSLKSEDTAVYYCAKNWRDAGTTWFEKSGSAGQGTQVTVSS

SEQ ID NO: 63 - protein, 118 aa, Lama glama
EVQLVESGGGLVQPGGSLRLSCAASGFTFSINTMGWYRQAPGKQRELVALISSIGDTYYADSVKGRFTISRDNAKNTVYLQMNSLKPEDTAVYYCKRFRTAAQGTDYWGQGTQVTVSS

SEQ ID NO: 64 - protein, 118 aa, Lama glama
EVQLVESGGGLVHPGGSLRLSCVGSGFSLDDYGMTWVRRAPGKGLEWVSSINWSGTHTDYADSVKGRFTISRDNAKNTLFLQMNSLNPEDTAVYYCGQGWKIVPTNPRGHGTQVTVSS

SEQ ID NO: 65 - protein, 118 aa, Lama glama
EVQLVESGGGLVQPGGSLRLSCVGSGFSLDDYAMTWVRQAPGKGLEWVSSINWSGTHTDYADSVKGRFTISRDNAKNTLFLQMNSLSPEDTAVYYCNQGWKIRPTIPMGHGTQVTVSS

SEQ ID NO: 66 - protein, 118 aa, Lama glama
EVQLVESGGGLVQPGGSLRLSCVASGFSLDDYGMTWVRQAPGKGLEWVSSINWSGTHTDYTDPVKGRFTISRDNAKNTLFLQMNNLTPEDTAVYYCNRGWKIVPTDLGGHGTQVTVSS

SEQ ID NO: 67 - protein, 122 aa, Lama glama
EVQLVESGGGLVQAGGSLRLSCAASGRTFISNYAMGWFRQAPGKEREFVATINWSGSHSDYADSVKGRFTISRDNAKNTVYLQMNNLKSEDTAVYYCAPGWGTAPLSTSVYWGQGTQVTVSS

SEQ ID NO: 68 - protein, 119 aa, Lama glama
EVQLVESGGGMVQAGGSLRLSCAASGLTLSNYGMGWFRQAPGKEREFVSSINWSGTHTYDADFVKGRFIISRDNAKNTVYLQINSLKPEDTAVYYCAAGGWGTGRYNYWGQGTQVTVSS

SEQ ID NO: 69 - protein, 119 aa, Lama glama; identical to SEQ ID NO: 68

SEQ ID NO: 70 - protein, 120 aa, Lama glama
EVQLVESGGGLVQAGGSLRLSCAASGRTFNAMGWFRQAPGKEREFVAAISRSPGVTYYADSVKGRFTTSRDNAKNTVYLQMNDLKPEDTAVYYCAADFYLATLAHEYDYWGQGTQVTVSS

SEQ ID NO: 71 - protein, 122 aa, Lama glama
EVQLVESGGGLVQAGGSLRLSCAASGRTFSSYAMAWFRQAPGTEREFIAGIRWSDGSTYYADSVKGRFTISRDNAKNTVYLQMNSLKPEDTAVYYCAADFYVSTLAHEYDYWGQGTQVTVSS

SEQ ID NO: 72 - protein, 122 aa, Lama glama
KVQLVESGGGLVQAGGSLRLSCAASGRTFSSYAMAWFRQAPGTEREFIAGIRWSDGSTYYADSVKGRFTISRANAKNTVYLQMNGLKPEDTAVYYCAADFYVSTLAHEYDYWGQGTQVTVSS